European Patent Specification EP 3 802 865 B1, published April 10, 2024. Title: Kit and method for the colorimetric detection of a target nucleic acid in a sample. Applicant: FONDAZIONE ISTITUTO ITALIANO DI TECNOLOGIA. The sequence listing filed with the application follows.

SEQUENCE LISTING (3 sequences)

SEQ ID NO: 1 - DNA, 28 bp, Artificial
  Probe P1
ccttccacaccttccaaacacacacaaa

SEQ ID NO: 2 - DNA, 43 bp, Artificial
  Probe P2
aaaaaaaaaaaaaaaaaaaaaaaaaaaaaatttaccactcaac

SEQ ID NO: 3 - DNA, 26 bp, Artificial
  Single strand synthetic sequence
aaggtgtggaagggttgagtggtaaa